European Patent Specification EP 4 058 604 B1, published April 22, 2026. Title: COMPOSITIONS AND METHODS FOR REGULATING EGFR AMPLIFICATION IN CANCER. Applicant: Fox Chase Cancer Center. The sequence listing filed with the application follows.

SEQUENCE LISTING (75 sequences)

SEQ ID NO: 1 - DNA, 21 bp, Homo sapiens
gaauagguauuggugaauutt

SEQ ID NO: 2 - DNA, 21 bp, Homo sapiens
ccauaaaugcuacgaauautt

SEQ ID NO: 3 - DNA, 21 bp, Homo sapiens
cuauggaagaguuccgaaatt

SEQ ID NO: 4 - DNA, 21 bp, Homo sapiens
gcgacaaucuuuauccugatt

SEQ ID NO: 5 - DNA, 21 bp, Homo sapiens
gcucuaacugaacaacuaatt

SEQ ID NO: 6 - DNA, 21 bp, Homo sapiens
cgcugauuuucgaguguaatt

SEQ ID NO: 7 - DNA, 21 bp, Homo sapiens
cagcugcaguaucucggaatt

SEQ ID NO: 8 - DNA, 21 bp, Homo sapiens
cucucaccguuuccacaaatt

SEQ ID NO: 9 - DNA, 21 bp, Homo sapiens
agaacagcuucgucauggatt

SEQ ID NO: 10 - DNA, 21 bp, Homo sapiens
caaaucgugugguacagaatt

SEQ ID NO: 11 - DNA, 21 bp, Homo sapiens
gaaugaguuuugucauggatt

SEQ ID NO: 12 - DNA, 21 bp, Homo sapiens
guauucgcuuugcaucuuutt

SEQ ID NO: 13 - DNA, 21 bp, Homo sapiens
ggacaaugcaggagauagatt

SEQ ID NO: 14 - DNA, 21 bp, Homo sapiens
caaccagacauauagaucatt

SEQ ID NO: 15 - DNA, 21 bp, Homo sapiens
gcugaccauugggacaguatt

SEQ ID NO: 16 - DNA, 21 bp, Homo sapiens
guguaugaguuuagagucatt

SEQ ID NO: 17 - DNA, 21 bp, Homo sapiens
ggaccgacauugguguauatt

SEQ ID NO: 18 - DNA, 21 bp, Homo sapiens
gcgaguuuguugugacauutt

SEQ ID NO: 19 - DNA, 21 bp, Homo sapiens
ggcaguaaaggaaaucgaatt

SEQ ID NO: 20 - DNA, 21 bp, Homo sapiens
ggaagaucuuggacuuauutt

SEQ ID NO: 21 - DNA, 21 bp, Homo sapiens
cagacgagagugaaacugatt

SEQ ID NO: 22 - DNA, 21 bp, Homo sapiens
ggaguuacuccauuaacuatt

SEQ ID NO: 23 - DNA, 21 bp, Homo sapiens
cagagaagcuagaccugaatt

SEQ ID NO: 24 - DNA, 21 bp, Homo sapiens
ggaguguaauaagugccgatt

SEQ ID NO: 25 - DNA, 21 bp, Homo sapiens
gguugcuauauguuccgaatt

SEQ ID NO: 26 - DNA, 21 bp, Homo sapiens
caacgacucaaaguauauatt

SEQ ID NO: 27 - DNA, 21 bp, Homo sapiens
cgcagugaguuugaacagatt

SEQ ID NO: 28 - DNA, 21 bp, Homo sapiens
cguucaaggcucaaccacatt

SEQ ID NO: 29 - DNA, 21 bp, Homo sapiens
cgguggaaauugucgaagatt

SEQ ID NO: 30 - DNA, 18 bp, Homo sapiens
gcctcccaccctatccaa

SEQ ID NO: 31 - DNA, 27 bp, Homo sapiens
tcatccagtgtgtatacatcatctctc

SEQ ID NO: 32 - DNA, 18 bp, Homo sapiens
ggcctcaagtgacgagga

SEQ ID NO: 33 - DNA, 20 bp, Homo sapiens
cttccactgcagagacagca

SEQ ID NO: 34 - DNA, 19 bp, Homo sapiens
agcagcagtgaagctgagg

SEQ ID NO: 35 - DNA, 24 bp, Homo sapiens
tgtacttaagcagctgtttcctga

SEQ ID NO: 36 - DNA, 18 bp, Homo sapiens
aatggcagacgtggtcgt

SEQ ID NO: 37 - DNA, 19 bp, Homo sapiens
tcttggctggagtctggag

SEQ ID NO: 38 - DNA, 22 bp, Homo sapiens
tcagcactgatacccaaacttc

SEQ ID NO: 39 - DNA, 23 bp, Homo sapiens
tcacatctccagattctgactga

SEQ ID NO: 40 - DNA, 21 bp, Homo sapiens
agcagactggcatctgtaagg

SEQ ID NO: 41 - DNA, 24 bp, Homo sapiens
gaagtttatcaacatcacatgcaa

SEQ ID NO: 42 - DNA, 21 bp, Homo sapiens
cgaacgcattgtttatcccta

SEQ ID NO: 43 - DNA, 21 bp, Homo sapiens
cgtgtgttacactgcacaagg

SEQ ID NO: 44 - DNA, 23 bp, Homo sapiens
ctgcacaagtaaaagcaactgtc

SEQ ID NO: 45 - DNA, 26 bp, Homo sapiens
cttttggagatactgaatagcatagc

SEQ ID NO: 46 - DNA, 19 bp, Homo sapiens
accctcgaaatcccatcac

SEQ ID NO: 47 - DNA, 18 bp, Homo sapiens
gtgttcgccactcgcttc

SEQ ID NO: 48 - DNA, 23 bp, Homo sapiens
gacagtgtgcgttatgtttgact

SEQ ID NO: 49 - DNA, 26 bp, Homo sapiens
tggccaatatatatagtaaacgacca

SEQ ID NO: 50 - DNA, 20 bp, Homo sapiens
ggaggaagcagcaagcagta

SEQ ID NO: 51 - DNA, 19 bp, Homo sapiens
gctcaggtttggggattgt

SEQ ID NO: 52 - DNA, 21 bp, Homo sapiens
ccacgaaaacaaagaggacag

SEQ ID NO: 53 - DNA, 24 bp, Homo sapiens
tgggtgcttacacttacacaagat

SEQ ID NO: 54 - DNA, 20 bp, Homo sapiens
atcctggagacacccatcag

SEQ ID NO: 55 - DNA, 19 bp, Homo sapiens
gacaggctcagggtcagtg

SEQ ID NO: 56 - DNA, 20 bp, Homo sapiens
gcggtcagagaacagctacc

SEQ ID NO: 57 - DNA, 20 bp, Homo sapiens
ggaggctgaagatgcagaga

SEQ ID NO: 58 - DNA, 19 bp, Homo sapiens
caagttcacggacgcctac

SEQ ID NO: 59 - DNA, 18 bp, Homo sapiens
ccgcgggagaattgtgta

SEQ ID NO: 60 - DNA, 20 bp, Homo sapiens
tgggaaaggtgacctcagat

SEQ ID NO: 61 - DNA, 21 bp, Homo sapiens
gggcagaacctaactcctctg

SEQ ID NO: 62 - DNA, 20 bp, Homo sapiens
gccaaagaggtgacgatagc

SEQ ID NO: 63 - DNA, 18 bp, Homo sapiens
actgcccgttgtggtgtc

SEQ ID NO: 64 - DNA, 21 bp, Homo sapiens
gtcatggagtacgtgggagag

SEQ ID NO: 65 - DNA, 20 bp, Homo sapiens
cctgacggtcgtagatctgg

SEQ ID NO: 66 - DNA, 23 bp, Homo sapiens
tctttcaaaaatgttgtcctgct

SEQ ID NO: 67 - DNA, 22 bp, Homo sapiens
aggtgggattttaatttgttgg

SEQ ID NO: 68 - DNA, 19 bp, Homo sapiens
gcttccccttccctctttc

SEQ ID NO: 69 - DNA, 21 bp, Homo sapiens
gggaagacatgcttttgtcct

SEQ ID NO: 70 - DNA, 22 bp, Homo sapiens
tgggaccaaaacatgtagacag

SEQ ID NO: 71 - DNA, 21 bp, Homo sapiens
ttccttggaggagtatccaca

SEQ ID NO: 72 - DNA, 21 bp, Homo sapiens
gatacagctcagaccccacag

SEQ ID NO: 73 - DNA, 19 bp, Homo sapiens
ttttgggaacggactggtt

SEQ ID NO: 74 - DNA, 17 bp, Homo sapiens
aggccaaccgcgagaag

SEQ ID NO: 75 - DNA, 23 bp, Homo sapiens
acagcctggatagcaacgtacat